European Patent Specification EP 3 426 284 B1, published May 8, 2024. Title: GLUCAGON AND GLP-1 CO-AGONISTS FOR THE TREATMENT OF OBESITY. Applicant: MedImmune LIMITED JERMUTUS, Lutz AMBERY, Philip Duncan BEDNAREK, Maria A. PETRONE, Marcella. The sequence listing filed with the application follows.

SEQUENCE LISTING (26 sequences)

SEQ ID NO: 1 - protein, 29 aa, Homo sapiens
HSQGTFTSDYSKYLDSRRAQDFVQWLMNT

SEQ ID NO: 2 - protein, 30 aa, Homo sapiens
HAEGTFTSDVSSYLEGQAAKEFIAWLVKGR

SEQ ID NO: 3 - protein, 31 aa, Homo sapiens
HAEGTFTSDVSSYLEGQAAKEFIAWLVKGRG

SEQ ID NO: 4 - protein, 30 aa, Artificial Sequence
  chimeric GLP-1/glucagon peptide
  MISC_FEATURE (2)..(2): Xaa is Gly or Ser
  MISC_FEATURE (10)..(10): Xaa is Tyr or Lys
  MISC_FEATURE (12)..(12): Xaa is Lys, Glu, Arg, or Ser
  MISC_FEATURE (13)..(13): Xaa is Lys or Tyr
  MISC_FEATURE (15)..(15): Xaa is Asp or Glu
  MISC_FEATURE (16)..(16): Xaa is Ser or Gly
  MISC_FEATURE (17)..(17): Xaa is Glu, Arg, Gln, or Lys
  MISC_FEATURE (18)..(18): Xaa is Arg, Ser, or Ala
  MISC_FEATURE (20)..(20): Xaa is Arg, Lys, or Gln
  MISC_FEATURE (21)..(21): Xaa is Asp or Glu
  MISC_FEATURE (23)..(23): Xaa is Val or Ile
  MISC_FEATURE (24)..(24): Xaa is Ala or Gln
  MISC_FEATURE (27)..(27): Xaa is Glu or Val
  MISC_FEATURE (28)..(28): Xaa is Ala or Lys
  MISC_FEATURE (30)..(30): Xaa is Gly or Arg
HXQGTFTSDXSXXLXXXXAXXFXXWLXXGX

SEQ ID NO: 5 - protein, 30 aa, Artificial Sequence
  chimeric GLP-1/glucagon peptide
  MISC_FEATURE (10)..(10): Xaa is Tyr or Lys
  MISC_FEATURE (12)..(12): Xaa is Lys, Glu, Arg, or Ser
  MISC_FEATURE (13)..(13): Xaa is Lys or Tyr
  MISC_FEATURE (17)..(17): Xaa is Glu, Arg, Gln, or Lys
  MISC_FEATURE (18)..(18): Xaa is Arg, Ser, or Ala
  MISC_FEATURE (27)..(27): Xaa is Glu or Val
HSQGTFTSDXSXXLDSXXARDFVAWLXAGG

SEQ ID NO: 6 - protein, 30 aa, Artificial Sequence
  chimeric GLP-1/glucagon peptide
  MISC_FEATURE (10)..(10): Xaa is Tyr or Lys
  MISC_FEATURE (12)..(12): Xaa is Lys, Glu, Arg, or Ser
  MISC_FEATURE (13)..(13): Xaa is Lys or Tyr
  MISC_FEATURE (27)..(27): Xaa is Glu or Val
HSQGTFTSDXSXXLDSERARDFVAWLXAGG

SEQ ID NO: 7 - protein, 30 aa, Artificial Sequence
  chimeric GLP-1/glucagon peptide
  MISC_FEATURE (10)..(10): Xaa is Tyr or Lys
  MISC_FEATURE (12)..(12): Xaa is Lys, Glu, Arg, or Ser
  MISC_FEATURE (13)..(13): Xaa is Lys or Tyr
  MISC_FEATURE (27)..(27): Xaa is Glu or Val
HSQGTFTSDXSXXLDSRSARDFVAWLXAGG

SEQ ID NO: 8 - protein, 30 aa, Artificial Sequence
  chimeric GLP-1/glucagon peptide
HSQGTFTSDYSKKLDSERARDFVAWLVAGG

SEQ ID NO: 9 - protein, 30 aa, Artificial Sequence
  chimeric GLP-1/glucagon peptide
HSQGTFTSDYSKKLDSRSARDFVAWLVAGG

SEQ ID NO: 10 - protein, 30 aa, Artificial Sequence
  chimeric GLP-1/glucagon peptide
  MISC_FEATURE (12)..(12): Xaa is Lys, Glu, or Arg
HSQGTFTSDKSXYLDSERARDFVAWLEAGG

SEQ ID NO: 11 - protein, 30 aa, Artificial Sequence
  chimeric GLP-1/glucagon peptide
  MISC_FEATURE (12)..(12): Xaa is Lys, Glu, Arg, or Ser
HSQGTFTSDKSXYLDSRSARDFVAWLEAGG

SEQ ID NO: 12 - protein, 30 aa, Artificial Sequence
  chimeric GLP-1/glucagon peptide
HSQGTFTSDKSEYLDSERARDFVAWLEAGG

SEQ ID NO: 13 - protein, 30 aa, Artificial Sequence
  chimeric GLP-1/glucagon peptide
HSQGTFTSDKSEYLDSRSARDFVAWLEAGG

SEQ ID NO: 14 - protein, 30 aa, Artificial Sequence
  chimeric GLP-1/glucagon peptide
HSQGTFTSDKSRYLDSERARDFVAWLEAGG

SEQ ID NO: 15 - protein, 30 aa, Artificial Sequence
  chimeric GLP-1/glucagon peptide
HSQGTFTSDKSRYLDSRSARDFVAWLEAGG

SEQ ID NO: 16 - protein, 30 aa, Artificial Sequence; identical to SEQ ID NO: 8
  chimeric GLP-1/glucagon peptide
  MISC_FEATURE (13)..(13): Lysine with a palmitoyl group conjugated to the epsilon nitrogen, through a gamma glutamic acid linker

SEQ ID NO: 17 - protein, 30 aa, Artificial Sequence; identical to SEQ ID NO: 12
  chimeric GLP-1/glucagon peptide
  MISC_FEATURE (10)..(10): Lysine with a palmitoyl group conjugated to the epsilon nitrogen, through a gamma glutamic acid linker

SEQ ID NO: 18 - protein, 30 aa, Artificial Sequence; identical to SEQ ID NO: 15
  chimeric GLP-1/glucagon peptide
  MISC_FEATURE (10)..(10): Lysine with a palmitoyl group conjugated to the epsilon nitrogen, through a gamma glutamic acid linker

SEQ ID NO: 19 - protein, 30 aa, Artificial Sequence; identical to SEQ ID NO: 12
  chimeric GLP-1/glucagon peptide
  MISC_FEATURE (10)..(10): Lysine with a palmitoyl group conjugated to the epsilon nitrogen, through a gamma glutamic acid linker

SEQ ID NO: 20 - protein, 30 aa, Artificial Sequence
  chimeric GLP-1/glucagon peptide
  MISC_FEATURE (10)..(10): Lysine with a palmitoyl group conjugated to the epsilon nitrogen, through a gamma glutamic acid linker
HSQGTFTSDKSSYLDSRSARDFVAWLEAGG

SEQ ID NO: 21 - protein, 30 aa, Artificial Sequence
  chimeric GLP-1/glucagon peptide
  MISC_FEATURE (10)..(10): Lysine with a palmitoyl group conjugated to the epsilon nitrogen, through a gamma glutamic acid linker
HSQGTFTSDKSSYLDSRRARDFVAWLEAGG

SEQ ID NO: 22 - protein, 30 aa, Artificial Sequence
  chimeric GLP-1/glucagon peptide
  MISC_FEATURE (10)..(10): Lysine with a palmitoyl group conjugated to the epsilon nitrogen, through a gamma glutamic acid linker
HSQGTFTSDKSKYLEGQAAKEFIAWLEKGR

SEQ ID NO: 23 - protein, 30 aa, Artificial Sequence
  chimeric GLP-1/glucagon peptide
  MISC_FEATURE (17)..(17): Lysine with a palmitoyl group conjugated to the epsilon nitrogen, through a gamma glutamic acid linker
HGQGTFTSDYSKYLDSKRAQDFVQWLVAGG

SEQ ID NO: 24 - protein, 30 aa, Artificial Sequence; identical to SEQ ID NO: 8
  G931
  MISC_FEATURE (13)..(13): Lysine with a palmitoyl group conjugated to the epsilon nitrogen, through a gamma glutamic acid linker

SEQ ID NO: 25 - protein, 30 aa, Artificial Sequence; identical to SEQ ID NO: 22
  G934
  MISC_FEATURE (10)..(10): Lysine with a palmitoyl group conjugated to the epsilon nitrogen, through a gamma glutamic acid linker

SEQ ID NO: 26 - protein, 30 aa, Artificial Sequence; identical to SEQ ID NO: 20
  G973
  MISC_FEATURE (10)..(10): Lysine with a palmitoyl group conjugated to the epsilon nitrogen, through a gamma glutamic acid linker